European Patent Application EP 4 245 768 A1, published September 20, 2023. Title: PHARMACEUTICAL COMPOSITION COMPRISING HUMAN INTERLEUKIN 2 VARIANT OR DERIVATIVE THEREOF AND USE THEREOF. Applicant: Jiangsu Hengrui Pharmaceuticals Co., Ltd.; Shanghai Hengrui Pharmaceutical Co., Ltd.; Shanghai Shengdi Pharmaceutical Co., Ltd. Application EP21891204.6. The sequence listing filed with the application follows.

SEQUENCE LISTING (12 sequences)

SEQ ID NO: 1 - protein, 134 aa, Homo sapiens
MAPTSSSTKKTQLQLEHLLLDLQMILNGINNYKNPKLTRMLTFKFYMPKKATELKHLQCLEEELKPLEEVLNLAQSKNFHLRPRDLISNINVIVLELKGSETTFMCEYADETATIVEFLNRWITFCQSIISTLT

SEQ ID NO: 2 - protein, 134 aa, Artificial Sequence
  Amino acid sequence of IL-2 variant (N26Q/N29S/N88R)
  DISULFID (59)..(106)
MAPTSSSTKKTQLQLEHLLLDLQMILQGISNYKNPKLTRMLTFKFYMPKKATELKHLQCLEEELKPLEEVLNLAQSKNFHLRPRDLISRINVIVLELKGSETTFMCEYADETATIVEFLNRWITFAQSIISTLT

SEQ ID NO: 3 - protein, 134 aa, Artificial Sequence
  Amino acid sequence of IL-2 variant (N26Q)
MAPTSSSTKKTQLQLEHLLLDLQMILQGINNYKNPKLTRMLTFKFYMPKKATELKHLQCLEEELKPLEEVLNLAQSKNFHLRPRDLISNINVIVLELKGSETTFMCEYADETATIVEFLNRWITFAQSIISTLT

SEQ ID NO: 4 - protein, 134 aa, Artificial Sequence
  Amino acid sequence of IL-2 variant (N29S)
MAPTSSSTKKTQLQLEHLLLDLQMILNGISNYKNPKLTRMLTFKFYMPKKATELKHLQCLEEELKPLEEVLNLAQSKNFHLRPRDLISNINVIVLELKGSETTFMCEYADETATIVEFLNRWITFAQSIISTLT

SEQ ID NO: 5 - protein, 134 aa, Artificial Sequence
  Amino acid sequence of IL-2 variant (Q11C/L132C)
MAPTSSSTKKTCLQLEHLLLDLQMILNGINNYKNPKLTRMLTFKFYMPKKATELKHLQCLEEELKPLEEVLNLAQSKNFHLRPRDLISNINVIVLELKGSETTFMCEYADETATIVEFLNRWITFAQSIISTCT

SEQ ID NO: 6 - protein, 134 aa, Artificial Sequence
  Amino acid sequence of IL-2 variant (L70C/P82C)
MAPTSSSTKKTQLQLEHLLLDLQMILNGINNYKNPKLTRMLTFKFYMPKKATELKHLQCLEEELKPLEEVCNLAQSKNFHLRCRDLISNINVIVLELKGSETTFMCEYADETATIVEFLNRWITFAQSIISTLT

SEQ ID NO: 7 - protein, 134 aa, Artificial Sequence
  Amino acid sequence of IL-2 variant (G27C/F78C)
MAPTSSSTKKTQLQLEHLLLDLQMILNCINNYKNPKLTRMLTFKFYMPKKATELKHLQCLEEELKPLEEVLNLAQSKNCHLRPRDLISNINVIVLELKGSETTFMCEYADETATIVEFLNRWITFAQSIISTLT

SEQ ID NO: 8 - protein, 134 aa, Artificial Sequence
  Amino acid sequence of IL-2 variant (N26Q/N29S/N88G)
MAPTSSSTKKTQLQLEHLLLDLQMILQGISNYKNPKLTRMLTFKFYMPKKATELKHLQCLEEELKPLEEVLNLAQSKNFHLRPRDLISGINVIVLELKGSETTFMCEYADETATIVEFLNRWITFAQSIISTLT

SEQ ID NO: 9 - protein, 134 aa, Artificial Sequence
  Amino acid sequence of IL-2 variant (N26Q/N29S/N88I)
MAPTSSSTKKTQLQLEHLLLDLQMILQGISNYKNPKLTRMLTFKFYMPKKATELKHLQCLEEELKPLEEVLNLAQSKNFHLRPRDLISIINVIVLELKGSETTFMCEYADETATIVEFLNRWITFAQSIISTLT

SEQ ID NO: 10 - protein, 134 aa, Artificial Sequence
  Amino acid sequence of IL-2 variant (N26Q/N29S/N88D)
MAPTSSSTKKTQLQLEHLLLDLQMILQGISNYKNPKLTRMLTFKFYMPKKATELKHLQCLEEELKPLEEVLNLAQSKNFHLRPRDLISDINVIVLELKGSETTFMCEYADETATIVEFLNRWITFAQSIISTLT

SEQ ID NO: 11 - protein, 134 aa, Artificial Sequence
  Amino acid sequence of IL-2 variant (N26Q/N30S/N88R)
MAPTSSSTKKTQLQLEHLLLDLQMILQGINSYKNPKLTRMLTFKFYMPKKATELKHLQCLEEELKPLEEVLNLAQSKNFHLRPRDLISRINVIVLELKGSETTFMCEYADETATIVEFLNRWITFAQSIISTLT

SEQ ID NO: 12 - protein, 134 aa, Artificial Sequence
  Amino acid sequence of IL-2 variant (N26Q/N29S/N71Q/N88R)
MAPTSSSTKKTQLQLEHLLLDLQMILQGISNYKNPKLTRMLTFKFYMPKKATELKHLQCLEEELKPLEEVLQLAQSKNFHLRPRDLISRINVIVLELKGSETTFMCEYADETATIVEFLNRWITFAQSIISTLT